European Patent Specification EP 3 297 649 B1, published October 11, 2023. Title: PEPTIDE OLIGONUCLEOTIDE CONJUGATES. Applicant: Sarepta Therapeutics, Inc. The sequence listing filed with the application follows.

SEQUENCE LISTING (15 sequences)

SEQ ID NO: 1 - protein, 7 aa, Artificial Sequence
  synthetic peptide; see specification for cysteine modifications
  MOD_RES (1)..(1): ACETYLATION
CRRRCRG

SEQ ID NO: 2 - protein, 8 aa, Artificial Sequence
  synthetic peptide; see specification for cysteine modifications
  MOD_RES (1)..(1): ACETYLATION
CRRRCRRG

SEQ ID NO: 3 - protein, 9 aa, Artificial Sequence
  synthetic peptide; see specification for cysteine modifications
  MOD_RES (1)..(1): ACETYLATION
CRRRCRRRG

SEQ ID NO: 4 - protein, 9 aa, Artificial Sequence
  synthetic peptide; see specification for cysteine modifications
  MOD_RES (1)..(1): ACETYLATION
CRRRRRRCG

SEQ ID NO: 5 - protein, 8 aa, Artificial Sequence
  synthetic peptide; see specification for cysteine modifications
  MOD_RES (1)..(1): ACETYLATION
CRRRRRCG

SEQ ID NO: 6 - protein, 7 aa, Artificial Sequence
  synthetic peptide; see specification for cysteine modifications
  MOD_RES (1)..(1): ACETYLATION
CRRRRCG

SEQ ID NO: 7 - protein, 6 aa, Artificial Sequence
  synthetic peptide; see specification for cysteine modifications
  MOD_RES (1)..(1): ACETYLATION
CRRRCG

SEQ ID NO: 8 - protein, 5 aa, Artificial Sequence
  synthetic peptide; see specification for cysteine modifications
  MOD_RES (1)..(1): ACETYLATION
CRRCG

SEQ ID NO: 9 - DNA, 18 bp, Artificial Sequence
  phosphorodiamidate-linked morpholino oligomer
  misc_feature (1)..(18): phosphorodiamidate-linked morpholino residues
gctattaccttaacccag

SEQ ID NO: 10 - DNA, 27 bp, Artificial Sequence
  Dystrophin outer forward primer
caatgtttctggatgcagactttgtgg

SEQ ID NO: 11 - DNA, 27 bp, Artificial Sequence
  Dystrophin outer reverse primer
gttcagcttcactctttatcttctgcc

SEQ ID NO: 12 - DNA, 21 bp, Artificial Sequence
  Dystrophin inner forward primer
cacatctttgatggtgtgagg

SEQ ID NO: 13 - DNA, 22 bp, Artificial Sequence
  Dystrophin inner reverse primer
caacttcagccatccatttctg

SEQ ID NO: 14 - DNA, 25 bp, Artificial Sequence
  phosphorodiamidate-linked morpholino oligomer
  misc_feature (1)..(25): phosphorodiamidate-linked morpholino residues
ggccaaacctcggcttacctgaaat

SEQ ID NO: 15 - protein, 7 aa, Artificial Sequence
  synthetic peptide
  MOD_RES (1)..(1): ACETYLATION
RRRRRRG